European Patent Application EP 4 617 379 A1, published September 17, 2025. Title: COMPOSITION FOR PRETREATMENT AND METHOD FOR PRETREATMENT OF TARGET SAMPLE OF NUCLEIC ACID DETECTION. Applicant: Yokogawa Electric Corporation. Application EP. The sequence listing filed with the application follows.

SEQUENCE LISTING (5 sequences)

SEQ ID NO: 1 - DNA, 24 bp, synthetic construct
  source 1..24: mol_type = other DNA
gagtggtttgaccttaacgtttga

SEQ ID NO: 2 - DNA, 20 bp, synthetic construct
  source 1..20: mol_type = other DNA
ttgtcggttgcaatgcaagt

SEQ ID NO: 3 - DNA, 16 bp, synthetic construct
  source 1..16: mol_type = other DNA
cctaccgaagcaaatg

SEQ ID NO: 4 - DNA, 23 bp, synthetic construct
  source 1..23: mol_type = other DNA
tcaactagttcagtatggacgac

SEQ ID NO: 5 - DNA, 20 bp, synthetic construct
  source 1..20: mol_type = other DNA
cctcatcaagaaaccactga